European Patent Specification EP 4 034 555 B1, published February 12, 2025. Title: DAP10/DAP12 FUSION POLYPEPTIDES. Applicant: King's College London. The sequence listing filed with the application follows.

SEQUENCE LISTING (86 sequences)

SEQ ID NO: 1 - protein, 93 aa, Artificial Sequence
  isolated
MIHLGHILFLLLLPVAAAQTTPGERSSLPAFYPGTSGSCSGCGSLSLPLLAGLVAADAVASLLIVGAVFLCARPRRSPAQEDGKVYINMPGRG

SEQ ID NO: 2 - protein, 75 aa, Artificial Sequence
  isolated
QTTPGERSSLPAFYPGTSGSCSGCGSLSLPLLAGLVAADAVASLLIVGAVFLCARPRRSPAQEDGKVYINMPGRG

SEQ ID NO: 3 - protein, 51 aa, Artificial Sequence
  isolated
QTTPGERSSLPAFYPGTSGSCSGCGSLSLPLLAGLVAADAVASLLIVGAVF

SEQ ID NO: 4 - protein, 71 aa, Artificial Sequence
  isolated
MIHLGHILFLLLLPVAAAQTTPGERSSLPAFYPGTSGSCSGCGSLSLPLLAGLVAADAVASLLIVGAVFLC

SEQ ID NO: 5 - protein, 53 aa, Artificial Sequence
  isolated
QTTPGERSSLPAFYPGTSGSCSGCGSLSLPLLAGLVAADAVASLLIVGAVFLC

SEQ ID NO: 6 - protein, 24 aa, Artificial Sequence
  isolated
LCARPRRSPAQEDGKVYINMPGRG

SEQ ID NO: 7 - protein, 45 aa, Artificial Sequence
  isolated
LLAGLVAADAVASLLIVGAVFLCARPRRSPAQEDGKVYINMPGRG

SEQ ID NO: 8 - protein, 21 aa, Artificial Sequence
  isolated
LLAGLVAADAVASLLIVGAVF

SEQ ID NO: 9 - protein, 113 aa, Artificial Sequence
  isolated
MGGLEPCSRLLLLPLLLAVSGLRPVQAQAQSDCSCSTVSPGVLAGIVMGDLVLTVLIALAVYFLGRLVPRGRGAAEAATRKQRITETESPYQELQGQRSDVYSDLNTQRPYYK

SEQ ID NO: 10 - protein, 92 aa, Artificial Sequence
  isolated
LRPVQAQAQSDCSCSTVSPGVLAGIVMGDLVLTVLIALAVYFLGRLVPRGRGAAEAATRKQRITETESPYQELQGQRSDVYSDLNTQRPYYK

SEQ ID NO: 11 - protein, 52 aa, Artificial Sequence
  isolated
YFLGRLVPRGRGAAEAATRKQRITETESPYQELQGQRSDVYSDLNTQRPYYK

SEQ ID NO: 12 - protein, 21 aa, Artificial Sequence
  isolated
GVLAGIVMGDLVLTVLIALAV

SEQ ID NO: 13 - protein, 40 aa, Artificial Sequence
  isolated
LRPVQAQAQSDCSCSTVSPGVLAGIVMGDLVLTVLIALAV

SEQ ID NO: 14 - protein, 216 aa, Artificial Sequence
  isolated
MGWIRGRRSRHSWEMSEFHNYNLDLKKSDFSTRWQKQRCPVVKSKCRENASPFFFCCFIAVAMGIRFIIMVAIWSAVFLNSLFNQEVQIPLTESYCGPCPKNWICYKNNCYQFFDESKNWYESQASCMSQNASLLKVYSKEDQDLLKLVKSYHWMGLVHIPTNGSWQWEDGSILSPNLLTIIEMQKGDCALYASSFKGYIENCSTPNTYICMQRTV

SEQ ID NO: 15 - protein, 144 aa, Artificial Sequence
  isolated
IWSAVFLNSLFNQEVQIPLTESYCGPCPKNWICYKNNCYQFFDESKNWYESQASCMSQNASLLKVYSKEDQDLLKLVKSYHWMGLVHIPTNGSWQWEDGSILSPNLLTIIEMQKGDCALYASSFKGYIENCSTPNTYICMQRTV

SEQ ID NO: 16 - protein, 135 aa, Artificial Sequence
  isolated
LFNQEVQIPLTESYCGPCPKNWICYKNNCYQFFDESKNWYESQASCMSQNASLLKVYSKEDQDLLKLVKSYHWMGLVHIPTNGSWQWEDGSILSPNLLTIIEMQKGDCALYASSFKGYIENCSTPNTYICMQRTV

SEQ ID NO: 17 - protein, 165 aa, Artificial Sequence
  isolated
PFFFCCFIAVAMGIRFIIMVAIWSAVFLNSLFNQEVQIPLTESYCGPCPKNWICYKNNCYQFFDESKNWYESQASCMSQNASLLKVYSKEDQDLLKLVKSYHWMGLVHIPTNGSWQWEDGSILSPNLLTIIEMQKGDCALYASSFKGYIENCSTPNTYICMQRTV

SEQ ID NO: 18 - protein, 3 aa, Artificial Sequence
  isolated
GSG

SEQ ID NO: 19 - protein, 5 aa, Artificial Sequence
  isolated
GSGGG

SEQ ID NO: 20 - protein, 4 aa, Artificial Sequence
  isolated
GSGG

SEQ ID NO: 21 - protein, 4 aa, Artificial Sequence
  isolated
SGGG

SEQ ID NO: 22 - protein, 5 aa, Artificial Sequence
  isolated
GGGGS

SEQ ID NO: 23 - protein, 20 aa, Artificial Sequence
  isolated
GGGGSGGGGSGGGGSGGGGS

SEQ ID NO: 24 - protein, 15 aa, Artificial Sequence
  isolated
GGGGSGGGGSGGGGS

SEQ ID NO: 25 - protein, 5 aa, Artificial Sequence
  isolated
GPPGS

SEQ ID NO: 26 - protein, 4 aa, Artificial Sequence
  isolated
GGGS

SEQ ID NO: 27 - protein, 5 aa, Artificial Sequence
  isolated
GGGGS

SEQ ID NO: 28 - protein, 3 aa, Artificial Sequence
  isolated
GYS

SEQ ID NO: 29 - protein, 2 aa, Artificial Sequence
  isolated
GS

SEQ ID NO: 30 - protein, 5 aa, Artificial Sequence
  isolated
SGGGG

SEQ ID NO: 31 - protein, 4 aa, Artificial Sequence
  isolated
SGGG

SEQ ID NO: 32 - protein, 3 aa, Artificial Sequence
  isolated
SGG

SEQ ID NO: 33 - protein, 4 aa, Artificial Sequence
  isolated
SGSG

SEQ ID NO: 34 - protein, 2 aa, Artificial Sequence
  isolated
SG

SEQ ID NO: 35 - protein, 5 aa, Artificial Sequence
  isolated
GGGGA

SEQ ID NO: 36 - protein, 4 aa, Artificial Sequence
  isolated
GGGA

SEQ ID NO: 37 - protein, 5 aa, Artificial Sequence
  isolated
EAAAK

SEQ ID NO: 38 - protein, 4 aa, Artificial Sequence
  isolated
RRKR

SEQ ID NO: 39 - protein, 19 aa, Artificial Sequence
  isolated
ATNFSLLKQAGDVEENPGP

SEQ ID NO: 40 - protein, 18 aa, Artificial Sequence
  isolated
EGRGSLLTCGDVEENPGP

SEQ ID NO: 41 - protein, 23 aa, Artificial Sequence
  isolated
SGSGATNFSLLKQAGDVEENPGP

SEQ ID NO: 42 - protein, 22 aa, Artificial Sequence
  isolated
SGSGEGRGSLLTCGDVEENPGP

SEQ ID NO: 43 - protein, 27 aa, Artificial Sequence
  isolated
RRKRSGSGATNFSLLKQAGDVEENPGP

SEQ ID NO: 44 - protein, 26 aa, Artificial Sequence
  isolated
RRKRSGSGEGRGSLLTCGDVEENPGP

SEQ ID NO: 45 - protein, 22 aa, Artificial Sequence
  isolated
VKQTLNFDLLKLAGDVESNPGP

SEQ ID NO: 46 - protein, 20 aa, Artificial Sequence
  isolated
QCTNYALLKLAGDVESNPGP

SEQ ID NO: 47 - protein, 6 aa, Artificial Sequence
  isolated
HHHHHH

SEQ ID NO: 48 - protein, 8 aa, Artificial Sequence
  isolated
DYKDDDDK

SEQ ID NO: 49 - protein, 15 aa, Artificial Sequence
  isolated
GLNDIFEAQKIEWHE

SEQ ID NO: 50 - protein, 14 aa, Artificial Sequence
  isolated
GKPIPNPLLGLDST

SEQ ID NO: 51 - protein, 9 aa, Artificial Sequence
  isolated
IPNPLLGLD

SEQ ID NO: 52 - protein, 10 aa, Artificial Sequence
  isolated
EQKLISEEDL

SEQ ID NO: 53 - protein, 31 aa, Artificial Sequence
  isolated
GLNDIFEAQKIEWHEGGHHHHHHDYKDDDDK

SEQ ID NO: 54 - protein, 31 aa, Artificial Sequence
  isolated
DYKDDDDKHHHHHHGGGLNDIFEAQKIEWHE

SEQ ID NO: 55 - protein, 21 aa, Artificial Sequence
  isolated
MALPVTALLLPLALLLHAARP

SEQ ID NO: 56 - protein, 42 aa, Artificial Sequence
  isolated
KRGRKKLLYIFKQPFMRPVQTTQEEDGCSCRFPEEEEGGCEL

SEQ ID NO: 57 - protein, 48 aa, Artificial Sequence
  isolated
QRRKYRSNKGESPVEPAEPCHYSCPREEEGSTIPIQEDYRKPEPACSP

SEQ ID NO: 58 - protein, 12 aa, Artificial Sequence
  isolated
EPKSCDKTHTCP

SEQ ID NO: 59 - protein, 45 aa, Artificial Sequence
  isolated
TTTPAPRPPTPAPTIASQPLSLRPEACRPAAGGAVHTRGLDFACD

SEQ ID NO: 60 - protein, 145 aa, Artificial Sequence
  isolated
MIHLGHILFLLLLPVAAAQTTPGERSSLPAFYPGTSGSCSGCGSLSLPLLAGLVAADAVASLLIVGAVFLCARPRRSPAQEDGKVYINMPGRGYFLGRLVPRGRGAAEAATRKQRITETESPYQELQGQRSDVYSDLNTQRPYYK

SEQ ID NO: 61 - protein, 132 aa, Artificial Sequence
  isolated
MALPVTALLLPLALLLHAARPDYKDDDDKQTTPGERSSLPAFYPGTSGSCSGCGSLSLPLLAGLVAADAVASLLIVGAVFYFLGRLVPRGRGAAEAATRKQRITETESPYQELQGQRSDVYSDLNTQRPYYK

SEQ ID NO: 62 - protein, 138 aa, Artificial Sequence
  isolated
MALPVTALLLPLALLLHAARPDYKDDDDKEPKSCDKTHTCPLLAGLVAADAVASLLIVGAVFLCARPRRSPAQEDGKVYINMPGRGYFLGRLVPRGRGAAEAATRKQRITETESPYQELQGQRSDVYSDLNTQRPYYK

SEQ ID NO: 63 - protein, 171 aa, Artificial Sequence
  isolated
MALPVTALLLPLALLLHAARPDYKDDDDKTTTPAPRPPTPAPTIASQPLSLRPEACRPAAGGAVHTRGLDFACDLLAGLVAADAVASLLIVGAVFLCARPRRSPAQEDGKVYINMPGRGYFLGRLVPRGRGAAEAATRKQRITETESPYQELQGQRSDVYSDLNTQRPYYK

SEQ ID NO: 64 - protein, 388 aa, Artificial Sequence
  isolated
MIHLGHILFLLLLPVAAAQTTPGERSSLPAFYPGTSGSCSGCGSLSLPLLAGLVAADAVASLLIVGAVFLCARPRRSPAQEDGKVYINMPGRGYFLGRLVPRGRGAAEAATRKQRITETESPYQELQGQRSDVYSDLNTQRPYYKRRKRSGSGATNFSLLKQAGDVEENPGPMGWIRGRRSRHSWEMSEFHNYNLDLKKSDFSTRWQKQRCPVVKSKCRENASPFFFCCFIAVAMGIRFIIMVAIWSAVFLNSLFNQEVQIPLTESYCGPCPKNWICYKNNCYQFFDESKNWYESQASCMSQNASLLKVYSKEDQDLLKLVKSYHWMGLVHIPTNGSWQWEDGSILSPNLLTIIEMQKGDCALYASSFKGYIENCSTPNTYICMQRTV

SEQ ID NO: 65 - protein, 494 aa, Artificial Sequence
  isolated
MALPVTALLLPLALLLHAARPDYKDDDDKQTTPGERSSLPAFYPGTSGSCSGCGSLSLPLLAGLVAADAVASLLIVGAVFYFLGRLVPRGRGAAEAATRKQRITETESPYQELQGQRSDVYSDLNTQRPYYKRRKRSGSGEGRGSLLTCGDVEENPGPMIHLGHILFLLLLPVAAAQTTPGERSSLPAFYPGTSGSCSGCGSLSLPLLAGLVAADAVASLLIVGAVFLCARPRRSPAQEDGKVYINMPGRGRRKRSGSGATNFSLLKQAGDVEENPGPMGWIRGRRSRHSWEMSEFHNYNLDLKKSDFSTRWQKQRCPVVKSKCRENASPFFFCCFIAVAMGIRFIIMVAIWSAVFLNSLFNQEVQIPLTESYCGPCPKNWICYKNNCYQFFDESKNWYESQASCMSQNASLLKVYSKEDQDLLKLVKSYHWMGLVHIPTNGSWQWEDGSILSPNLLTIIEMQKGDCALYASSFKGYIENCSTPNTYICMQRTV

SEQ ID NO: 66 - protein, 527 aa, Artificial Sequence
  isolated
MIHLGHILFLLLLPVAAAQTTPGERSSLPAFYPGTSGSCSGCGSLSLPLLAGLVAADAVASLLIVGAVFLCARPRRSPAQEDGKVYINMPGRGYFLGRLVPRGRGAAEAATRKQRITETESPYQELQGQRSDVYSDLNTQRPYYKRRKRSGSGATNFSLLKQAGDVEENPGPMGWIRGRRSRHSWEMSEFHNYNLDLKKSDFSTRWQKQRCPVVKSKCRENASPFFFCCFIAVAMGIRFIIMVAIWSAVFLNSLFNQEVQIPLTESYCGPCPKNWICYKNNCYQFFDESKNWYESQASCMSQNASLLKVYSKEDQDLLKLVKSYHWMGLVHIPTNGSWQWEDGSILSPNLLTIIEMQKGDCALYASSFKGYIENCSTPNTYICMQRTVRRKRSGSGEGRGSLLTCGDVEENPGPMIHLGHILFLLLLPVAAAQTTPGERSSLPAFYPGTSGSCSGCGSLSLPLLAGLVAADAVASLLIVGAVFLCKRGRKKLLYIFKQPFMRPVQTTQEEDGCSCRFPEEEEGGCEL

SEQ ID NO: 67 - protein, 538 aa, Artificial Sequence
  isolated
MIHLGHILFLLLLPVAAAQTTPGERSSLPAFYPGTSGSCSGCGSLSLPLLAGLVAADAVASLLIVGAVFLCARPRRSPAQEDGKVYINMPGRGYFLGRLVPRGRGAAEAATRKQRITETESPYQELQGQRSDVYSDLNTQRPYYKRRKRSGSGATNFSLLKQAGDVEENPGPMGWIRGRRSRHSWEMSEFHNYNLDLKKSDFSTRWQKQRCPVVKSKCRENASPFFFCCFIAVAMGIRFIIMVAIWSAVFLNSLFNQEVQIPLTESYCGPCPKNWICYKNNCYQFFDESKNWYESQASCMSQNASLLKVYSKEDQDLLKLVKSYHWMGLVHIPTNGSWQWEDGSILSPNLLTIIEMQKGDCALYASSFKGYIENCSTPNTYICMQRTVRRKRSGSGEGRGSLLTCGDVEENPGPMALPVTALLLPLALLLHAARPDYKDDDDKQTTPGERSSLPAFYPGTSGSCSGCGSLSLPLLAGLVAADAVASLLIVGAVFLCKRGRKKLLYIFKQPFMRPVQTTQEEDGCSCRFPEEEEGGCEL

SEQ ID NO: 68 - protein, 533 aa, Artificial Sequence
  isolated
MIHLGHILFLLLLPVAAAQTTPGERSSLPAFYPGTSGSCSGCGSLSLPLLAGLVAADAVASLLIVGAVFLCARPRRSPAQEDGKVYINMPGRGYFLGRLVPRGRGAAEAATRKQRITETESPYQELQGQRSDVYSDLNTQRPYYKRRKRSGSGATNFSLLKQAGDVEENPGPMGWIRGRRSRHSWEMSEFHNYNLDLKKSDFSTRWQKQRCPVVKSKCRENASPFFFCCFIAVAMGIRFIIMVAIWSAVFLNSLFNQEVQIPLTESYCGPCPKNWICYKNNCYQFFDESKNWYESQASCMSQNASLLKVYSKEDQDLLKLVKSYHWMGLVHIPTNGSWQWEDGSILSPNLLTIIEMQKGDCALYASSFKGYIENCSTPNTYICMQRTVRRKRSGSGEGRGSLLTCGDVEENPGPMIHLGHILFLLLLPVAAAQTTPGERSSLPAFYPGTSGSCSGCGSLSLPLLAGLVAADAVASLLIVGAVFLCQRRKYRSNKGESPVEPAEPCHYSCPREEEGSTIPIQEDYRKPEPACSP

SEQ ID NO: 69 - protein, 544 aa, Artificial Sequence
  isolated
MIHLGHILFLLLLPVAAAQTTPGERSSLPAFYPGTSGSCSGCGSLSLPLLAGLVAADAVASLLIVGAVFLCARPRRSPAQEDGKVYINMPGRGYFLGRLVPRGRGAAEAATRKQRITETESPYQELQGQRSDVYSDLNTQRPYYKRRKRSGSGATNFSLLKQAGDVEENPGPMGWIRGRRSRHSWEMSEFHNYNLDLKKSDFSTRWQKQRCPVVKSKCRENASPFFFCCFIAVAMGIRFIIMVAIWSAVFLNSLFNQEVQIPLTESYCGPCPKNWICYKNNCYQFFDESKNWYESQASCMSQNASLLKVYSKEDQDLLKLVKSYHWMGLVHIPTNGSWQWEDGSILSPNLLTIIEMQKGDCALYASSFKGYIENCSTPNTYICMQRTVRRKRSGSGEGRGSLLTCGDVEENPGPMALPVTALLLPLALLLHAARPDYKDDDDKQTTPGERSSLPAFYPGTSGSCSGCGSLSLPLLAGLVAADAVASLLIVGAVFLCQRRKYRSNKGESPVEPAEPCHYSCPREEEGSTIPIQEDYRKPEPACSP

SEQ ID NO: 70 - DNA, 435 bp, Artificial Sequence
  isolated
atgatccacctgggccacatcctgttcctgctgctgctgcccgtggccgctgcccagaccacccctggcgagcggagcagcctgcctgccttctaccctggcaccagcggcagctgcagcggctgcggcagcctgagcctgcccctgctggccggcctggtggccgccgacgccgtggccagcctgctgatcgtgggcgccgtgttcctgtgcgccaggcccaggcggagccctgcccaggaggacggcaaggtgtacatcaacatgcccggccggggctacttcctgggcaggctggtgcccaggggcaggggcgctgccgaggctgccacccggaagcagcggatcaccgagaccgagagcccctaccaggagctgcagggccagcggagcgacgtgtacagcgacctgaacacccagaggccctactacaag

SEQ ID NO: 71 - DNA, 396 bp, Artificial Sequence
  isolated
atggctctgcctgtgacagctctgctgctgcctctggctctgctgctgcacgccgctagacccgattataaggacgacgacgacaagcagaccacccctggcgagcggagcagcctgcctgccttctaccctggcaccagcggcagctgcagcggctgcggcagcctgagcctgcccctgctggctggcctggtggccgccgacgccgtggccagcctgctgatcgtgggcgccgtgttctacttcctgggcaggctggtgcccaggggcaggggcgctgccgaggctgccacccggaagcagcggatcaccgagaccgagagcccctaccaggagctgcagggccagcggagcgacgtgtacagcgacctgaacacccagaggccctactacaag

SEQ ID NO: 72 - DNA, 414 bp, Artificial Sequence
  isolated
atggctctgcctgtgacagctctgctgctgcctctggctctgctgctgcacgccgctagacccgattataaggacgacgacgacaaggagcccaagagctgcgacaagacacacacatgccctcttctggccggcctggtggccgccgacgccgtggccagcctgctgatcgtgggcgccgtgttcctgtgcgccaggcccaggcggagccctgcccaggaggacggcaaggtgtacatcaacatgcccggccggggctacttcctgggcaggctggtgcccaggggcaggggcgctgccgaggctgccacccggaagcagcggatcaccgagaccgagagcccctaccaggagctgcagggccagcggagcgacgtgtacagcgacctgaacacccagaggccctactacaag

SEQ ID NO: 73 - DNA, 513 bp, Artificial Sequence
  isolated
atggctctgcctgtgacagctctgctgctgcctctggctctgctgctgcacgccgctagacccgattataaggacgacgacgacaagaccacaacacctgctcctagacctcccacccctgctcccaccatcgccagccagcccctgagcctgagacccgaggcctgcagacccgctgctggcggcgctgtgcataccagaggcctggatttcgcctgcgaccttctggccggcctggtggccgccgacgccgtggccagcctgctgatcgtgggcgccgtgttcctgtgcgccaggcccaggcggagccctgcccaggaggacggcaaggtgtacatcaacatgcccggccggggctacttcctgggcaggctggtgcccaggggcaggggcgctgccgaggctgccacccggaagcagcggatcaccgagaccgagagcccctaccaggagctgcagggccagcggagcgacgtgtacagcgacctgaacacccagaggccctactacaag

SEQ ID NO: 74 - DNA, 1164 bp, Artificial Sequence
  isolated
atgatccacctgggccacatcctgttcctgctgctgctgcccgtggccgctgcccagaccacccctggcgagcggagcagcctgcctgccttctaccctggcaccagcggcagctgcagcggctgcggcagcctgagcctgcccctgctggccggcctggtggccgccgacgccgtggccagcctgctgatcgtgggcgccgtgttcctgtgcgccaggcccaggcggagccctgcccaggaggacggcaaggtgtacatcaacatgcccggccggggctacttcctgggcaggctggtgcccaggggcaggggcgctgccgaggctgccacccggaagcagcggatcaccgagaccgagagcccctaccaggagctgcagggccagcggagcgacgtgtacagcgacctgaacacccagaggccctactacaagaggcggaaaaggtctgggagtggggctaccaatttctctctcctcaagcaagccggagacgttgaggaaaaccctggacccatgggctggatccggggacggaggagccggcacagctgggagatgagcgagttccacaactacaacctggacctgaagaagagcgacttcagcacccggtggcagaagcagcggtgccccgtggtgaagagcaagtgccgggagaacgccagccccttcttcttctgctgcttcatcgccgtggctatgggcatccggttcatcatcatggtggccatctggagcgccgtgttcctgaacagcctgttcaaccaggaggtgcagatccccctgaccgagagctactgcggcccctgccccaagaactggatctgctacaagaacaactgctaccagttcttcgacgagagcaagaactggtacgagagccaggccagctgcatgagccagaacgccagcctgctgaaggtgtacagcaaggaggaccaggacctgctgaagctggtgaagagctaccactggatgggcctggtgcacatccccaccaacggcagctggcagtgggaggacggcagcatcctgagccccaacctgctgaccatcatcgagatgcagaagggcgactgcgccctgtacgccagcagcttcaagggctacatcgagaactgcagcacccccaacacctacatctgcatgcagcggaccgtg

SEQ ID NO: 75 - DNA, 1482 bp, Artificial Sequence
  isolated
atggctctgcctgtgacagctctgctgctgcctctggctctgctgctgcacgccgctagacccgattataaggacgacgacgacaagcagaccacccctggcgagcggagcagcctgcctgccttctaccctggcaccagcggcagctgcagcggctgcggcagcctgagcctgcccctgctggctggcctggtggccgccgacgccgtggccagcctgctgatcgtgggcgccgtgttctacttcctgggcaggctggtgcccaggggcaggggcgctgccgaggctgccacccggaagcagcggatcaccgagaccgagagcccctaccaggagctgcagggccagcggagcgacgtgtacagcgacctgaacacccagaggccctactacaagcggagaaagcgctccggctccggcgagggccgcggcagcctgctgacctgcggcgacgtggaagagaaccccggacccatgatccacctgggccacatcctgttcctgctgctgctgcccgtggccgctgcccaaacaacacccggcgagagatcctccttgcccgctttctatcccggaacatccggaagctgttccggatgtggatccctttctttgcctttgcttgctggattggtcgcagctgacgctgtcgcttccctccttattgtcggagctgtcttcctgtgcgccaggcccaggcggagccctgcccaggaggacggcaaggtgtacatcaacatgcccggccggggcaggcggaagcgctccgggagtggggctaccaatttctctctcctcaagcaagccggagacgttgaggaaaaccctggacccatgggctggatccggggacggaggagccggcacagctgggagatgagcgagttccacaactacaacctggacctgaagaagagcgacttcagcacccggtggcagaagcagcggtgccccgtggtgaagagcaagtgccgggagaacgccagccccttcttcttctgctgcttcatcgccgtggctatgggcatccggttcatcatcatggtggccatctggagcgccgtgttcctgaacagcctgttcaaccaggaggtgcagatccccctgaccgagagctactgcggcccctgccccaagaactggatctgctacaagaacaactgctaccagttcttcgacgagagcaagaactggtacgagagccaggccagctgcatgagccagaacgccagcctgctgaaggtgtacagcaaggaggaccaggacctgctgaagctggtgaagagctaccactggatgggcctggtgcacatccccaccaacggcagctggcagtgggaggacggcagcatcctgagccccaacctgctgaccatcatcgagatgcagaagggcgactgcgccctgtacgccagcagcttcaagggctacatcgagaactgcagcacccccaacacctacatctgcatgcagcggaccgtg

SEQ ID NO: 76 - DNA, 1581 bp, Artificial Sequence
  isolated
atgatccacctgggccacatcctgttcctgctgctgctgcccgtggccgctgcccagaccacccctggcgagcggagcagcctgcctgccttctaccctggcaccagcggcagctgcagcggctgcggcagcctgagcctgcccctgctggccggcctggtggccgccgacgccgtggccagcctgctgatcgtgggcgccgtgttcctgtgcgccaggcccaggcggagccctgcccaggaggacggcaaggtgtacatcaacatgcccggccggggctacttcctgggcaggctggtgcccaggggcaggggcgctgccgaggctgccacccggaagcagcggatcaccgagaccgagagcccctaccaggagctgcagggccagcggagcgacgtgtacagcgacctgaacacccagaggccctactacaagaggcggaaaaggtctgggagtggggctaccaatttctctctcctcaagcaagccggagacgttgaggaaaaccctggacccatgggctggatccggggacggaggagccggcacagctgggagatgagcgagttccacaactacaacctggacctgaagaagagcgacttcagcacccggtggcagaagcagcggtgccccgtggtgaagagcaagtgccgggagaacgccagccccttcttcttctgctgcttcatcgccgtggctatgggcatccggttcatcatcatggtggccatctggagcgccgtgttcctgaacagcctgttcaaccaggaggtgcagatccccctgaccgagagctactgcggcccctgccccaagaactggatctgctacaagaacaactgctaccagttcttcgacgagagcaagaactggtacgagagccaggccagctgcatgagccagaacgccagcctgctgaaggtgtacagcaaggaggaccaggacctgctgaagctggtgaagagctaccactggatgggcctggtgcacatccccaccaacggcagctggcagtgggaggacggcagcatcctgagccccaacctgctgaccatcatcgagatgcagaagggcgactgcgccctgtacgccagcagcttcaagggctacatcgagaactgcagcacccccaacacctacatctgcatgcagcggaccgtgagaagaaagagaagcggcagcggcgagggcagaggcagcctgctgacctgcggcgacgtggaggagaaccccggacccatgattcatctcggacatattctctttctcttgctcttgcctgtcgctgccgctcaaacaactcccggagaaagatcttctctccccgctttttatcccggaacatctggatcttgttctggatgtggatctttgtctctccctctcctcgctggactcgtcgcagctgatgctgtcgcttctctcttgattgtcggagctgtctttttgtgtaagagaggcagaaagaagctgctgtacatcttcaagcagcccttcatgagacccgtgcagaccacccaggaggaggacggctgcagctgcagattccccgaggaggaggagggcggctgcgagctg

SEQ ID NO: 77 - DNA, 1614 bp, Artificial Sequence
  isolated
atgatccacctgggccacatcctgttcctgctgctgctgcccgtggccgctgcccagaccacccctggcgagcggagcagcctgcctgccttctaccctggcaccagcggcagctgcagcggctgcggcagcctgagcctgcccctgctggccggcctggtggccgccgacgccgtggccagcctgctgatcgtgggcgccgtgttcctgtgcgccaggcccaggcggagccctgcccaggaggacggcaaggtgtacatcaacatgcccggccggggctacttcctgggcaggctggtgcccaggggcaggggcgctgccgaggctgccacccggaagcagcggatcaccgagaccgagagcccctaccaggagctgcagggccagcggagcgacgtgtacagcgacctgaacacccagaggccctactacaagaggcggaaaaggtctgggagtggggctaccaatttctctctcctcaagcaagccggagacgttgaggaaaaccctggacccatgggctggatccggggacggaggagccggcacagctgggagatgagcgagttccacaactacaacctggacctgaagaagagcgacttcagcacccggtggcagaagcagcggtgccccgtggtgaagagcaagtgccgggagaacgccagccccttcttcttctgctgcttcatcgccgtggctatgggcatccggttcatcatcatggtggccatctggagcgccgtgttcctgaacagcctgttcaaccaggaggtgcagatccccctgaccgagagctactgcggcccctgccccaagaactggatctgctacaagaacaactgctaccagttcttcgacgagagcaagaactggtacgagagccaggccagctgcatgagccagaacgccagcctgctgaaggtgtacagcaaggaggaccaggacctgctgaagctggtgaagagctaccactggatgggcctggtgcacatccccaccaacggcagctggcagtgggaggacggcagcatcctgagccccaacctgctgaccatcatcgagatgcagaagggcgactgcgccctgtacgccagcagcttcaagggctacatcgagaactgcagcacccccaacacctacatctgcatgcagcggaccgtgagaagaaagagaagcggcagcggcgagggcagaggcagcctgctgacctgcggcgacgtggaggagaaccccggacctatggctctgcctgtgacagctctgctgctgcctctggctctgctgctgcacgccgctagacccgattataaggacgacgacgacaagcaaacaactcccggagaaagatcttctctccccgctttttatcccggaacatctggatcttgttctggatgtggatctttgtctctccctctcctcgctggactcgtcgcagctgatgctgtcgcttctctcttgattgtcggagctgtctttttgtgtaagagaggcagaaagaagctgctgtacatcttcaagcagcccttcatgagacccgtgcagaccacccaggaggaggacggctgcagctgcagattccccgaggaggaggagggcggctgcgagctg

SEQ ID NO: 78 - DNA, 1599 bp, Artificial Sequence
  isolated
atgatccacctgggccacatcctgttcctgctgctgctgcccgtggccgctgcccagaccacccctggcgagcggagcagcctgcctgccttctaccctggcaccagcggcagctgcagcggctgcggcagcctgagcctgcccctgctggccggcctggtggccgccgacgccgtggccagcctgctgatcgtgggcgccgtgttcctgtgcgccaggcccaggcggagccctgcccaggaggacggcaaggtgtacatcaacatgcccggccggggctacttcctgggcaggctggtgcccaggggcaggggcgctgccgaggctgccacccggaagcagcggatcaccgagaccgagagcccctaccaggagctgcagggccagcggagcgacgtgtacagcgacctgaacacccagaggccctactacaagaggcggaaaaggtctgggagtggggctaccaatttctctctcctcaagcaagccggagacgttgaggaaaaccctggacccatgggctggatccggggacggaggagccggcacagctgggagatgagcgagttccacaactacaacctggacctgaagaagagcgacttcagcacccggtggcagaagcagcggtgccccgtggtgaagagcaagtgccgggagaacgccagccccttcttcttctgctgcttcatcgccgtggctatgggcatccggttcatcatcatggtggccatctggagcgccgtgttcctgaacagcctgttcaaccaggaggtgcagatccccctgaccgagagctactgcggcccctgccccaagaactggatctgctacaagaacaactgctaccagttcttcgacgagagcaagaactggtacgagagccaggccagctgcatgagccagaacgccagcctgctgaaggtgtacagcaaggaggaccaggacctgctgaagctggtgaagagctaccactggatgggcctggtgcacatccccaccaacggcagctggcagtgggaggacggcagcatcctgagccccaacctgctgaccatcatcgagatgcagaagggcgactgcgccctgtacgccagcagcttcaagggctacatcgagaactgcagcacccccaacacctacatctgcatgcagcggaccgtgagaagaaagagaagcggcagcggcgagggcagaggcagcctgctgacctgcggcgacgtggaggagaaccccggacccatgattcatctcggacatattctctttctcttgctcttgcctgtcgctgccgctcaaacaactcccggagaaagatcttctctccccgctttttatcccggaacatctggatcttgttctggatgtggatctttgtctctccctctcctcgctggactcgtcgcagctgatgctgtcgcttctctcttgattgtcggagctgtctttttgtgtcagaggcggaagtaccggagcaacaagggcgagagccccgtggagcctgccgagccctgccactacagctgtccccgggaggaggagggcagcaccatccccatccaggaggactaccggaagcccgagcctgcctgcagcccc

SEQ ID NO: 79 - DNA, 1632 bp, Artificial Sequence
  isolated
atgatccacctgggccacatcctgttcctgctgctgctgcccgtggccgctgcccagaccacccctggcgagcggagcagcctgcctgccttctaccctggcaccagcggcagctgcagcggctgcggcagcctgagcctgcccctgctggccggcctggtggccgccgacgccgtggccagcctgctgatcgtgggcgccgtgttcctgtgcgccaggcccaggcggagccctgcccaggaggacggcaaggtgtacatcaacatgcccggccggggctacttcctgggcaggctggtgcccaggggcaggggcgctgccgaggctgccacccggaagcagcggatcaccgagaccgagagcccctaccaggagctgcagggccagcggagcgacgtgtacagcgacctgaacacccagaggccctactacaagaggcggaaaaggtctgggagtggggctaccaatttctctctcctcaagcaagccggagacgttgaggaaaaccctggacccatgggctggatccggggacggaggagccggcacagctgggagatgagcgagttccacaactacaacctggacctgaagaagagcgacttcagcacccggtggcagaagcagcggtgccccgtggtgaagagcaagtgccgggagaacgccagccccttcttcttctgctgcttcatcgccgtggctatgggcatccggttcatcatcatggtggccatctggagcgccgtgttcctgaacagcctgttcaaccaggaggtgcagatccccctgaccgagagctactgcggcccctgccccaagaactggatctgctacaagaacaactgctaccagttcttcgacgagagcaagaactggtacgagagccaggccagctgcatgagccagaacgccagcctgctgaaggtgtacagcaaggaggaccaggacctgctgaagctggtgaagagctaccactggatgggcctggtgcacatccccaccaacggcagctggcagtgggaggacggcagcatcctgagccccaacctgctgaccatcatcgagatgcagaagggcgactgcgccctgtacgccagcagcttcaagggctacatcgagaactgcagcacccccaacacctacatctgcatgcagcggaccgtgagaagaaagagaagcggcagcggcgagggcagaggcagcctgctgacctgcggcgacgtggaggagaaccccggacctatggctctgcctgtgacagctctgctgctgcctctggctctgctgctgcacgccgctagacccgattataaggacgacgacgacaagcaaacaactcccggagaaagatcttctctccccgctttttatcccggaacatctggatcttgttctggatgtggatctttgtctctccctctcctcgctggactcgtcgcagctgatgctgtcgcttctctcttgattgtcggagctgtctttttgtgtcagaggcggaagtaccggagcaacaagggcgagagccccgtggagcctgccgagccctgccactacagctgtccccgggaggaggagggcagcaccatccccatccaggaggactaccggaagcccgagcctgcctgcagcccc

SEQ ID NO: 80 - protein, 20 aa, Artificial Sequence
  isolated
NAVPNLRGDLQVLAQKVART

SEQ ID NO: 81 - protein, 25 aa, Artificial Sequence
  isolated
MGWLCSGLLFPVSCLVLLQVASSGN

SEQ ID NO: 82 - protein, 107 aa, Artificial Sequence
  isolated
IEVMYPPPYLDNEKSNGTIIHVKGKHLCPSPLFPGPSKPFWVLVVVGGVLACYSLLVTVAFIIFWVRSKRSRLLHSDYMNMTPRRPGPTRKHYQPYAPPRDFAAYRS

SEQ ID NO: 83 - protein, 112 aa, Artificial Sequence
  isolated
RVKFSRSADAPAYQQGQNQLYNELNLGRREEYDVLDKRRGRDPEMGGKPRRKNPQEGLYNELQKDKMAEAYSEIGMKGERRRGKGHDGLYQGLSTATKDTYDALHMQALPPR

SEQ ID NO: 84 - protein, 695 aa, Artificial Sequence
  isolated
MGWSCIILFLVATATGVHSQIQLVQSGPELKKPGETVKISCKTSGYTFTDYSMHWVNQAPGKGLKWMGWINTETGEPTYTDDFKGRFAFSLETSASTAYLQINNLKNEDTATYFCARTAVYWGQGTTLTVSSGSTSGSGKPGSGEGSDIQMTQSPSSLSASLGERVSLTCRASQEISGSLSWLQQKPDGTIKRLIYAASTLNSGVPKRFSGRRSGSDYSLTISSLESEDFVDYYCLQYSSYPWSFGGGTKLEIKEPKSPDKTHTCPPCPSHTQPLGVFLFPPKPKDQLMISRTPEVTCVVVDVSQEDPEVQFNWYVDGVEVHNAKTKPREEQFNSTYRVVSVLTVLHQDWLNGKEYKCKVSNKGLPSSIEKTISKAKGQPREPQVYTLPPSQEEMTKNQVSLTCLVKGFYPSDIAVEWESNGQPENNYKTTPPVLDSDGSFFLYSRLTVDKSRWQEGNVFSCSVLHEALHNHYTQKSLSLSLGKFWVLVVVGGVLACYSLLVTVAFIIFWVARPRRSPAQEDGKVYINMPGRGGRLVPRGRGAAEAATRKQRITETESPYQELQGQRSDVYSDLNTQRPYYKRVKFSRSADAPAYQQGQNQLYNELNLGRREEYDVLDKRRGRDPEMGGKPQRRKNPQEGLYNELQKDKMAEAYSEIGMKGERRRGKGHDGLYQGLSTATKDTYDALHMQALPPR

SEQ ID NO: 85 - protein, 22 aa, Artificial Sequence
  isolated
ARPRRSPAQEDGKVYINMPGRG

SEQ ID NO: 86 - protein, 49 aa, Artificial Sequence
  isolated
GRLVPRGRGAAEAATRKQRITETESPYQELQGQRSDVYSDLNTQRPYYK